European Patent Application EP 4 538 369 A1, published April 16, 2025. Title: Hyaluronidase polypeptide and use thereof. Applicant: BMI Korea co., Ltd. The sequence listing filed with the application follows.

SEQUENCE LISTING (7 sequences)

SEQ ID NO: 1 - protein, 518 aa, synthetic construct
  REGION 1..518: note = Hyaluronidase (Example 1-1)
LDFRAPPLISNTSFLWAWNAPAERCVKIFKLPPDLRLFSVKGSPQKSATGQFITLFYADRLGYYPHIDEKTGNTVYGGIPQLGNLKNHLEKAKKDIAYYIPNDSVGLAVIDWENWRPTWARNWKPKDVYRDESVELVLQKNPQLSFPEASKIAKVDFETAGKSFMQETLKLGKLLRPNHLWGYYLFPDCYNHNYNQPTYNGNCSDLEKRRNDDLDWLWKESTALFPSVYLNIKLKSTPKAAFYVRNRVQEAIRLSKIASVESPLPVFVYHRPVFTDGSSTYLSQGDLVNSVGEIVALGASGIIMWGSLNLSLTMQSCMNLGNYLNTTLNPYIINVTLAAKMCSQVLCHDEGVCTRKQWNSSDYLHLNPMNFAIQTGKGGKYTVPGKVTLEDLQTFSDKFYCSCYANINCKKRVDIKNVHSVNVCMAEDICIEGPVKLQPSDHSSSQNEASTTTVSSISPSTTATTVSPCTPEKQSPECLKVRCLEAIANVTQTGCQGVKWKNTSSQSSIQNIKNQTTY

SEQ ID NO: 2 - protein, 483 aa, synthetic construct
  REGION 1..483: note = Hyaluronidase (Example 1-2)
DFRAPPLISNTSFLWAWNAPAERCVKIFKLPPDLRLFSVKGSPQKSATGQFITLFYADRLGYYPHIDEKTGNTVYGGIPQLGNLKNHLEKAKKDIAYYIPNDSVGLAVIDWENWRPTWARNWKPKDVYRDESVELVLQKNPQLSFPEASKIAKVDFETAGKSFMQETLKLGKLLRPNHLWGYYLFPDCYNHNYNQPTYNGNCSDLEKRRNDDLDWLWKESTALFPSVYLNIKLKSTPKAAFYVRNRVQEAIRLSKIASVESPLPVFVYHRPVFTDGSSTYLSQGDLVNSVGEIVALGASGIIMWGSLNLSLTMQSCMNLGNYLNTTLNPYIINVTLAAKMCSQVLCHDEGVCTRKQWNSSDYLHLNPMNFAIQTGKGGKYTVPGKVTLEDLQTFSDKFYCSCYANINCKKRVDIKNVHSVNVCMAEDICIEGPVKLQPSDHSSSQNEASTTTVSSISPSTTATTVSPCTPEKQSPECLKVRCL

SEQ ID NO: 3 - protein, 449 aa, synthetic construct
  REGION 1..449: note = Hyaluronidase (Example 1-3)
DFRAPPLISNTSFLWAWNAPAERCVKIFKLPPDLRLFSVKGSPQKSATGQFITLFYADRLGYYPHIDEKTGNTVYGGIPQLGNLKNHLEKAKKDIAYYIPNDSVGLAVIDWENWRPTWARNWKPKDVYRDESVELVLQKNPQLSFPEASKIAKVDFETAGKSFMQETLKLGKLLRPNHLWGYYLFPDCYNHNYNQPTYNGNCSDLEKRRNDDLDWLWKESTALFPSVYLNIKLKSTPKAAFYVRNRVQEAIRLSKIASVESPLPVFVYHRPVFTDGSSTYLSQGDLVNSVGEIVALGASGIIMWGSLNLSLTMQSCMNLGNYLNTTLNPYIINVTLAAKMCSQVLCHDEGVCTRKQWNSSDYLHLNPMNFAIQTGKGGKYTVPGKVTLEDLQTFSDKFYCSCYANINCKKRVDIKNVHSVNVCMAEDICIEGPVKLQPSDHSSSQNEAS

SEQ ID NO: 4 - protein, 415 aa, synthetic construct
  REGION 1..415: note = Hyaluronidase (Example 1-4)
DFRAPPLISNTSFLWAWNAPAERCVKIFKLPPDLRLFSVKGSPQKSATGQFITLFYADRLGYYPHIDEKTGNTVYGGIPQLGNLKNHLEKAKKDIAYYIPNDSVGLAVIDWENWRPTWARNWKPKDVYRDESVELVLQKNPQLSFPEASKIAKVDFETAGKSFMQETLKLGKLLRPNHLWGYYLFPDCYNHNYNQPTYNGNCSDLEKRRNDDLDWLWKESTALFPSVYLNIKLKSTPKAAFYVRNRVQEAIRLSKIASVESPLPVFVYHRPVFTDGSSTYLSQGDLVNSVGEIVALGASGIIMWGSLNLSLTMQSCMNLGNYLNTTLNPYIINVTLAAKMCSQVLCHDEGVCTRKQWNSSDYLHLNPMNFAIQTGKGGKYTVPGKVTLEDLQTFSDKFYCSCYANINCKKRVDIK

SEQ ID NO: 5 - protein, 381 aa, synthetic construct
  REGION 1..381: note = Hyaluronidase (Example 1-5)
DFRAPPLISNTSFLWAWNAPAERCVKIFKLPPDLRLFSVKGSPQKSATGQFITLFYADRLGYYPHIDEKTGNTVYGGIPQLGNLKNHLEKAKKDIAYYIPNDSVGLAVIDWENWRPTWARNWKPKDVYRDESVELVLQKNPQLSFPEASKIAKVDFETAGKSFMQETLKLGKLLRPNHLWGYYLFPDCYNHNYNQPTYNGNCSDLEKRRNDDLDWLWKESTALFPSVYLNIKLKSTPKAAFYVRNRVQEAIRLSKIASVESPLPVFVYHRPVFTDGSSTYLSQGDLVNSVGEIVALGASGIIMWGSLNLSLTMQSCMNLGNYLNTTLNPYIINVTLAAKMCSQVLCHDEGVCTRKQWNSSDYLHLNPMNFAIQTGKGGKYT

SEQ ID NO: 6 - protein, 347 aa, synthetic construct
  REGION 1..347: note = Hyaluronidase (Example 1-6)
DFRAPPLISNTSFLWAWNAPAERCVKIFKLPPDLRLFSVKGSPQKSATGQFITLFYADRLGYYPHIDEKTGNTVYGGIPQLGNLKNHLEKAKKDIAYYIPNDSVGLAVIDWENWRPTWARNWKPKDVYRDESVELVLQKNPQLSFPEASKIAKVDFETAGKSFMQETLKLGKLLRPNHLWGYYLFPDCYNHNYNQPTYNGNCSDLEKRRNDDLDWLWKESTALFPSVYLNIKLKSTPKAAFYVRNRVQEAIRLSKIASVESPLPVFVYHRPVFTDGSSTYLSQGDLVNSVGEIVALGASGIIMWGSLNLSLTMQSCMNLGNYLNTTLNPYIINVTLAAKMCSQVLCH

SEQ ID NO: 7 - protein, 313 aa, synthetic construct
  REGION 1..313: note = Hyaluronidase (Example 1-7)
DFRAPPLISNTSFLWAWNAPAERCVKIFKLPPDLRLFSVKGSPQKSATGQFITLFYADRLGYYPHIDEKTGNTVYGGIPQLGNLKNHLEKAKKDIAYYIPNDSVGLAVIDWENWRPTWARNWKPKDVYRDESVELVLQKNPQLSFPEASKIAKVDFETAGKSFMQETLKLGKLLRPNHLWGYYLFPDCYNHNYNQPTYNGNCSDLEKRRNDDLDWLWKESTALFPSVYLNIKLKSTPKAAFYVRNRVQEAIRLSKIASVESPLPVFVYHRPVFTDGSSTYLSQGDLVNSVGEIVALGASGIIMWGSLNLSLTM